European Patent Application EP 4 342 988 A1, published March 27, 2024. Title: Compositions and methods for modification of the expression of a SNCA gene. Applicant: Eberhard Karls Universität Tübingen - Medizinische Fakultät. Application EP. The sequence listing filed with the application follows.

SEQUENCE LISTING (60 sequences)

SEQ ID NO: 1 - DNA, 1560 bp, synthetic construct
  source 1..1560: mol_type = other DNA
aatttcctggatgctcagtggttagctaagtcttaagtttatgaatgaacaaatgacacaagatacaacattagaacgaggatggagaaaaaatataaaatctttaaaatatcagtcaaacgacaaattccagcttcttatgaatgaagagccagttaaatacgtttgaatgaaaaatgacgtgtgaagtgatatatgtggcagttaaagttaaccaggagagaaagctaaactaccgctgcacaggctcagcatctattgcactaatctaggcatgagttgtgtcctatccaaaccttcataatggaagagatgggggagagaatgaaagagagattggaaaaaacaaggatcctaaaatcatcttatggctaaatttgagagggagggaactatggaggcatcagtgatttatatggtttatattgtaggtcatgggaagtcataagaaaaattctggtgccaatggtgataactgatatgaagggactccttgcttgaaggaaaaattaagttaaactgagacctgttgaaatcaaagtagtagtgtgatatctaaataaaaatgtgtagcgtgcaaagagaaatatgagagtgtgtatcaggcaagagatctggctagaaatgtaggcaaagggataaatagtcataagactataaggcattgcggagggaagaggaaaagcttggagaatgagtcagaaatccacacaatagattaaagatttaagttgtgagaaagtttttatggagagtgttctggggaataaattagagattaataaaagaataaaaaatcaaccaggtagaaagggcatgcatcctggtgtgtgcaaacatgtatagctgcatgaatgtcaagtttactatcttacgtggctatatcactatgcaaactatagcctttcatagtacgtaagtgaaagcattagaggattatctgtgtagtcctaaaatcctttgtgaatacatcacattgtcctattacattcttgcccatgttttacataaccagactgactgtaatatgagtattgtgtgtgccctttgttaataaatccttgtataaaccccacaaggatttctctaaagacaaacctggcttgctaaatattactcactccaggctaaattttaataaattccataaaacactatcagatatattcctgagacttttgtattttaagtgctgtcttttcctatttggtatttgcattggttacttttgtggggtgtgctggtttcttccttcttccccttcagacactccaccccactcctgcactgtgcctggagaagatgaattgtactgactacaccacggtttttcaaccttggcagtaatgacattttttaactggatactttgttgtggaaggatgtcctgtgcattgtagatgtttaaaaaaatccctcagtgaatcatagtagcactccactcctctcccttcctcccctgagctgtgataaccactaatgttccctgggagcacaattggccctggattagaaccactgctacatcaatgcactccttttgtctacgctgtgagtttg

SEQ ID NO: 2 - DNA, 1401 bp, synthetic construct
  source 1..1401: mol_type = other DNA
gtatctggcacatttggggttataaatcacaaataacataaataagataatgttaatctccttcttacaaaatccaatggcttcccacaagtctatatataatatgcaaatttcttactatagcttataagatctggaataatttttcctatctccagccttcacctcttctcacattcatcatattctagctaatcaggactcttttatgtcataaaatatgctagatttgcacacccttaaagccttcatatacgagtttgttctgccttggatacctctgttccacattcccgaacattctctctctcatcacacagctggaccctttcaccctcctgatctcaattgaaatgtgaccttcctgtataaactttccatgagctggcttgtctgactgaacccaaatggctaatggattttctttcccgttacatgctctctaatttatgatgctttgcttggggggaaaatgagaggtgggagtctgtttacggaacatggaagtccttttgcagaggtacaagagtggaaatggctgttccccagcctggctctctgagtcagacctgacatccacagagagagcactgcagtaactgcaaacgcttctgttttgattgtggtaattggaacaatcagggcacaaactgcaaggtcactggcaagggtagcagcaggcatgattcctcccttagtaattttaaagcagcagatttcaaaagggaaaaccaagcagatgaaagtgagcagatttgttcttcagcacatgtgagatacccttggagatgccaataaatcactggagagactgtgaaggaggcttaggccctgcagatgaagttagtgatggagggaaatcgtgtttatcctcgggctgtcaggtctgaaatacctgggttaagtaaatggcctctgggatggtcacagtcggcaattattagcagttacagatccatctctatgccaaaacagataacagcatccaggaattatccaaagtcacaaatcagtgtcagtgtcttgtcactcacccacgtagtgcttttcccttcctcctagttacttaatggataagggcacattgtcaaataaacaaacaagtgaggataaatgttgctccgaaatttaaggtgaatcattagtcagacttggtatcgtcatggaatttggtctgttttctaactagctttattttagcacagccataaatctggctgtaattgtctttaactccgatgactcatacatctaagcatttcatttaactttcaaccgtgaaaaattccaactgatttggcaatatgaatgtgctcttacatgcatatgatcatatgatgctgtcagtacaacatctgtttttgttcttgggatgttgatggactatcatgaaccatctta

SEQ ID NO: 3 - DNA, 20 bp, synthetic construct
  source 1..20: mol_type = other DNA
gggcgagaatagtcaatatc

SEQ ID NO: 4 - DNA, 20 bp, synthetic construct
  source 1..20: mol_type = other DNA
gatcaagtttgtctaacccg

SEQ ID NO: 5 - DNA, 20 bp, synthetic construct
  source 1..20: mol_type = other DNA
gccatattgtgtagcaacag

SEQ ID NO: 6 - DNA, 20 bp, synthetic construct
  source 1..20: mol_type = other DNA
tcttgatagcttctaagtca

SEQ ID NO: 7 - DNA, 20 bp, synthetic construct
  source 1..20: mol_type = other DNA
ctgataccacctgcctgcac

SEQ ID NO: 8 - DNA, 20 bp, synthetic construct
  source 1..20: mol_type = other DNA
gcatggtcacaacttactaa

SEQ ID NO: 9 - DNA, 21 bp, synthetic construct
  source 1..21: mol_type = other DNA
gacgtatcagaaagaggttat

SEQ ID NO: 10 - DNA, 21 bp, synthetic construct
  source 1..21: mol_type = other DNA
gcctgtaaaggagtttcattt

SEQ ID NO: 11 - DNA, 21 bp, synthetic construct
  source 1..21: mol_type = other DNA
ggaatctcattcgatgcatac

SEQ ID NO: 12 - DNA, 20 bp, synthetic construct
  source 1..20: mol_type = other DNA
gaaagacttaccagagacgc

SEQ ID NO: 13 - DNA, 22 bp, synthetic construct
  source 1..22: mol_type = other DNA
gcctaattcattcaccaaaggg

SEQ ID NO: 14 - DNA, 20 bp, synthetic construct
  source 1..20: mol_type = other DNA
ggtgtggcatatcatgggtt

SEQ ID NO: 15 - DNA, 20 bp, synthetic construct
  source 1..20: mol_type = other DNA
ggtgatgaacttggggtcga

SEQ ID NO: 16 - DNA, 20 bp, synthetic construct
  source 1..20: mol_type = other DNA
ttcttctccactaggcccaa

SEQ ID NO: 17 - DNA, 20 bp, synthetic construct
  source 1..20: mol_type = other DNA
ctctggggaggaactcagaa

SEQ ID NO: 18 - DNA, 20 bp, synthetic construct
  source 1..20: mol_type = other DNA
gtgctactatgattcactga

SEQ ID NO: 19 - DNA, 20 bp, synthetic construct
  source 1..20: mol_type = other DNA
gacgtgtgaagtgatatatg

SEQ ID NO: 20 - DNA, 20 bp, synthetic construct
  source 1..20: mol_type = other DNA
caaactcacagcgtagacaa

SEQ ID NO: 21 - DNA, 20 bp, synthetic construct
  source 1..20: mol_type = other DNA
aatttcctggatgctcagtg

SEQ ID NO: 22 - DNA, 20 bp, synthetic construct
  source 1..20: mol_type = other DNA
tcttgatagcttctaagtca

SEQ ID NO: 23 - DNA, 20 bp, synthetic construct
  source 1..20: mol_type = other DNA
ttgcatttgcgtatttgtgc

SEQ ID NO: 24 - DNA, 20 bp, synthetic construct
  source 1..20: mol_type = other DNA
acttggctgaatctgagtcc

SEQ ID NO: 25 - DNA, 20 bp, synthetic construct
  source 1..20: mol_type = other DNA
gggaatattggtgagcatgg

SEQ ID NO: 26 - DNA, 20 bp, synthetic construct
  source 1..20: mol_type = other DNA
ggatctaaggaccctcaaca

SEQ ID NO: 27 - DNA, 20 bp, synthetic construct
  source 1..20: mol_type = other DNA
cctcatgaatggctttgagt

SEQ ID NO: 28 - DNA, 20 bp, synthetic construct
  source 1..20: mol_type = other DNA
aagccaagtagcaattcagg

SEQ ID NO: 29 - DNA, 26 bp, synthetic construct
  source 1..26: mol_type = other DNA
ggccaaaatgaactaaatgaacaggg

SEQ ID NO: 30 - DNA, 26 bp, synthetic construct
  source 1..26: mol_type = other DNA
gaacttggctgaatctgagtccattc

SEQ ID NO: 31 - DNA, 26 bp, synthetic construct
  source 1..26: mol_type = other DNA
cgtatatgaaggctttaagggtgtgc

SEQ ID NO: 32 - DNA, 22 bp, synthetic construct
  source 1..22: mol_type = other DNA
agctagcaaaggctttctgcta

SEQ ID NO: 33 - DNA, 22 bp, synthetic construct
  source 1..22: mol_type = other DNA
tctcgagggtggaaaggcagaa

SEQ ID NO: 34 - DNA, 20 bp, synthetic construct
  source 1..20: mol_type = other DNA
taaaggggactgggaaagtt

SEQ ID NO: 35 - DNA, 20 bp, synthetic construct
  source 1..20: mol_type = other DNA
aaaaccatcaccacagttcc

SEQ ID NO: 36 - DNA, 20 bp, synthetic construct
  source 1..20: mol_type = other DNA
aatgcactggaaaggttgtt

SEQ ID NO: 37 - DNA, 20 bp, synthetic construct
  source 1..20: mol_type = other DNA
tctttttccccatgaggtct

SEQ ID NO: 38 - DNA, 20 bp, synthetic construct
  source 1..20: mol_type = other DNA
ggaaaatggtgatagtggcg

SEQ ID NO: 39 - DNA, 20 bp, synthetic construct
  source 1..20: mol_type = other DNA
tgagggtgaaagggagacta

SEQ ID NO: 40 - DNA, 20 bp, synthetic construct
  source 1..20: mol_type = other DNA
ttcatcttctccaggcacag

SEQ ID NO: 41 - DNA, 20 bp, synthetic construct
  source 1..20: mol_type = other DNA
ggttacttttgtggggtgtg

SEQ ID NO: 42 - DNA, 20 bp, synthetic construct
  source 1..20: mol_type = other DNA
aataattgccgactgtgacc

SEQ ID NO: 43 - DNA, 20 bp, synthetic construct
  source 1..20: mol_type = other DNA
gtgatggagggaaatcgtgt

SEQ ID NO: 44 - DNA, 20 bp, synthetic construct
  source 1..20: mol_type = other DNA
gctgagaaaaccaaacaggg

SEQ ID NO: 45 - DNA, 20 bp, synthetic construct
  source 1..20: mol_type = other DNA
gaacaagcaccaaactgaca

SEQ ID NO: 46 - DNA, 20 bp, synthetic construct
  source 1..20: mol_type = other DNA
gtcaaaaaggaccagttggg

SEQ ID NO: 47 - DNA, 20 bp, synthetic construct
  source 1..20: mol_type = other DNA
ccaggcctcacatgaaaatg

SEQ ID NO: 48 - DNA, 22 bp, synthetic construct
  source 1..22: mol_type = other DNA
gtctatgccctgtttagcaatc

SEQ ID NO: 49 - DNA, 22 bp, synthetic construct
  source 1..22: mol_type = other DNA
tcttaccctgtaggactttcat

SEQ ID NO: 50 - DNA, 20 bp, synthetic construct
  source 1..20: mol_type = other DNA
aagcagcaggaaagacaaaa

SEQ ID NO: 51 - DNA, 20 bp, synthetic construct
  source 1..20: mol_type = other DNA
acatctgtcagcagatctca

SEQ ID NO: 52 - DNA, 20 bp, synthetic construct
  source 1..20: mol_type = other DNA
ctgtggatcctgacaatgag

SEQ ID NO: 53 - DNA, 20 bp, synthetic construct
  source 1..20: mol_type = other DNA
caagaaactgggagcaaaga

SEQ ID NO: 54 - DNA, 20 bp, synthetic construct
  source 1..20: mol_type = other DNA
agaaggagattactgccctg

SEQ ID NO: 55 - DNA, 20 bp, synthetic construct
  source 1..20: mol_type = other DNA
ccaccaatccacacagagta

SEQ ID NO: 56 - DNA, 20 bp, synthetic construct
  source 1..20: mol_type = other DNA
acgaatggtcgtgggcaccg

SEQ ID NO: 57 - DNA, 20 bp, synthetic construct
  source 1..20: mol_type = other DNA
cctctcttgggccccttctg

SEQ ID NO: 58 - DNA, 84 bp, synthetic construct
  source 1..84: mol_type = other DNA
aatgatacggcgaccaccgagatctacactctttccctacacgacgctcttccgatctnnnnnnacgaatggtcgtgggcaccg

SEQ ID NO: 59 - DNA, 43 bp, synthetic construct
  source 1..43: mol_type = other DNA
caagcagaagacggcatacgagatgccgtcctcctcctcctag

SEQ ID NO: 60 - DNA, 17 bp, synthetic construct
  source 1..17: mol_type = other DNA
ggagggggtggtgctgc